European Patent Application EP 4 549 551 A1, published May 7, 2025. Title: The method for the generation of immortalized intestinal epithelial cells. Applicant: VILNIUS UNIVERSITY. Application EP. The sequence listing filed with the application follows.

SEQUENCE LISTING (2 sequences)

SEQ ID NO: 1 - RNA, 20 nt, synthetic construct
  source 1..20: mol_type = other RNA
gcgctgcgtcgtgcaccggg

SEQ ID NO: 2 - RNA, 20 nt, synthetic construct
  source 1..20: mol_type = other RNA
cccggtgcacgacgcagcgc